European Patent Application EP 4 491 719 A1, published January 15, 2025. Title: Methods of amplifying template nucleic acid using a thermostable TthPrimPol. Applicant: 4basebio, S.L.U. Application EP. The sequence listing filed with the application follows.

SEQUENCE LISTING (8 sequences)

SEQ ID NO: 1 - protein, 294 aa, Thermus thermophilus
MRPIEHVLGYARLGYAVLPLLPGEKRPHPRLVPHGLKEASRDPATLEAWWRSCPQAGAGILPAPEVLVLDFDDPEAWERLKEEHPTLLEAPRARTPRGGVHVYLRLPPEAVGRLSASVRAIPGVDLRGLGRSYLVAPPTTLPTGAYVWEVPLRRPEELPPVPAPLLARLLPPPPPPREVWTPVEGVSPKRLQALLQAYAAQVAHTPEGQRHNTLIRYAVAAGGLLPHGLDPREAEEALVAAAMSAGLPEAEARAAARWGLEVGASRPLALEPSLAPSGPRTYRARVYARMRRWA

SEQ ID NO: 2 - protein, 293 aa, Thermus thermophilus
MRPIEHALSYAAQGYGVLPLRPGGKEPLGKLVPHGLKNASRDPATLEAWWRSCPRCGVGILPGPEVLVLDFDDPEAWEGLRQEHPALEAAPRQRTPKGGRHVFLRLPEGVRLSASVRAIPGVDLRGMGRAYVVAAPTRLKDGRTYTWEAPLTPPEELPPVPQALLLKLLPPPPPPRPSWGAVGTASPKRLQALLQAYAAQVARTPEGQRHLTLIRYAVAAGGLIPHGLDPREAEEVLVAAAMSAGLPEWEARDAVRWGLGVGASRPLVLESSSKPPEPRTYRARVYARMRRWV

SEQ ID NO: 3 - DNA, 60 bp, synthetic construct
  source 1..60: mol_type = other DNA
ttttttttttttttttttttacgacagactnttttttttttttttttttttttttttttt

SEQ ID NO: 4 - DNA, 60 bp, synthetic construct
  source 1..60: mol_type = other DNA
ttttttttttttttttttttttttttttttttttttcctgtttttttttttttttttttt

SEQ ID NO: 5 - DNA, 29 bp, synthetic construct
  source 1..29: mol_type = other DNA
tttttttttttttttactntttttttttt

SEQ ID NO: 6 - DNA, 29 bp, synthetic construct
  source 1..29: mol_type = other DNA
tttttttttttttttcctctttttttttt

SEQ ID NO: 7 - DNA, 28 bp, synthetic construct
  source 1..28: mol_type = other DNA
agaagtgtatctggtactcactgtgatc

SEQ ID NO: 8 - DNA, 15 bp, synthetic construct
  source 1..15: mol_type = other DNA
gatcacagtgagtac